European Patent Application EP 4 549 464 A1, published May 7, 2025. Title: METHOD FOR PREPARING HER2 NANOBODY AND CONJUGATE, AND USE THEREOF. Applicant: FUDAN UNIVERSITY. Application US PCT/CN2023/101129, filed June 19, 2023. The sequence listing filed with the application follows.

SEQUENCE LISTING (27 sequences)

SEQ ID NO: 1 - protein, 8 aa, synthetic construct
  source 1..8: note = 1-C10 CDR1
GLTFRRYE

SEQ ID NO: 2 - protein, 8 aa, synthetic construct
  source 1..8: note = 1-C10 CDR2
ITPASGSR

SEQ ID NO: 3 - protein, 14 aa, synthetic construct
  source 1..14: note = 1-C10 CDR3
NAYWMIPQHIENNY

SEQ ID NO: 4 - protein, 121 aa, synthetic construct
  source 1..121: note = 1-C10 VH
QVQLVESGGDLVQPGGSLRLSCATSGLTFRRYELKWYRQAPGKERELVAGITPASGSRNYADSVKGRFTISRDDAKMTVYLQMNSLEPEDTAVYYCNAYWMIPQHIENNYWGKGTLVTVSS

SEQ ID NO: 5 - protein, 8 aa, synthetic construct
  source 1..8: note = 2-C07 CDR1
GLTFMRYD

SEQ ID NO: 6 - protein, 8 aa, synthetic construct
  source 1..8: note = 2-C07 CDR2
LDSSSGRT

SEQ ID NO: 7 - protein, 11 aa, synthetic construct
  source 1..11: note = 2-C07 CDR3
NAQWKRIGADY

SEQ ID NO: 8 - protein, 118 aa, synthetic construct
  source 1..118: note = 2-C07 VH
AVQLVESGGGLVQPGGSLRLSCAASGLTFMRYDINWYRQAPGKERELVAALDSSSGRTNYADFTEGRFTISRNNAKNSAYLQMNNLKPEDTASYYCNAQWKRIGADYWGQGTQVTVFS

SEQ ID NO: 9 - protein, 8 aa, synthetic construct
  source 1..8: note = 1-B05 CDR1
GITFFRHT

SEQ ID NO: 10 - protein, 8 aa, synthetic construct
  source 1..8: note = 1-B05 CDR2
ITGGESTN

SEQ ID NO: 11 - protein, 11 aa, synthetic construct
  source 1..11: note = 1-B05 CDR3
NSKWDAAGVEF

SEQ ID NO: 12 - protein, 114 aa, synthetic construct
  source 1..114: note = 1-B05 VH
AVQLVESGGGPGGSLRLSCAASGITFFRHTLGWYRQAPGKQRELVASITGGESTNYADSVKSRFTISRDNAKNMVFLQMNSLKPEDTALYYCNSKWDAAGVEFWGKGTLVTVSS

SEQ ID NO: 13 - protein, 8 aa, synthetic construct
  source 1..8: note = 1-C09 CDR1
GLTFRRYH

SEQ ID NO: 14 - protein, 8 aa, synthetic construct
  source 1..8: note = 1-C09 CDR2
ISDTGSTT

SEQ ID NO: 15 - protein, 11 aa, synthetic construct
  source 1..11: note = 1-C09 CDR3
NAKWPIIAADW

SEQ ID NO: 16 - protein, 118 aa, synthetic construct
  source 1..118: note = 1-C09 VH
DVQLVESGGGLVQPGGSLRLSCEASGLTFRRYHFSWYRQPPGKERELVAVISDTGSTTNYTDSVKGRFTISRDLARNTVFLQLNSLKPDDTAVYYCNAKWPIIAADWWGQGTQVTVSS

SEQ ID NO: 17 - protein, 8 aa, synthetic construct
  source 1..8: note = 2-F03 CDR1
GLTFRRYH

SEQ ID NO: 18 - protein, 8 aa, synthetic construct
  source 1..8: note = 2-F03 CDR2
ISDTGTTN

SEQ ID NO: 19 - protein, 11 aa, synthetic construct
  source 1..11: note = 2-F03 CDR3
NGRWPAVAADW

SEQ ID NO: 20 - protein, 117 aa, synthetic construct
  source 1..117: note = 2-F03 VH
EVQLVESGGGLVQPGGSLRLSCAASGLTFRRYHMSWYRQAPGKERELVAVISDTGTTNYAESVKGRFTISRDNSRSTVFLQLNSLKPDDTAVYYCNGRWPAVAADWWGQGTQVTVSS

SEQ ID NO: 21 - protein, 8 aa, synthetic construct
  source 1..8: note = 1-G07 CDR1
RITFRHYD

SEQ ID NO: 22 - protein, 8 aa, synthetic construct
  source 1..8: note = 1-G07 CDR2
VTNGGVIT

SEQ ID NO: 23 - protein, 19 aa, synthetic construct
  source 1..19: note = 1-G07 CDR3
NAVWVYLQRLTQNKKENDY

SEQ ID NO: 24 - protein, 125 aa, synthetic construct
  source 1..125: note = 1-G07 VH
QVQLVESGGGKAQPGGSLRLSCVASRITFRHYDLSWYRQAPGQERELVATVTNGGVITYADSVKGRFTISRDNAKNTVQLQMNNLKPEDTAVYYCNAVWVYLQRLTQNKKENDYWGPGTQVTVSS

SEQ ID NO: 25 - protein, 357 aa, synthetic construct
  source 1..357: note = 1-G07-FC1
QVQLVESGGGKAQPGGSLRLSCVASRITFRHYDLSWYRQAPGQERELVATVTNGGVITYADSVKGRFTISRDNAKNTVQLQMNNLKPEDTAVYYCNAVWVYLQRLTQNKKENDYWGPGTQVTVSSEPKSSDKTHTCPPCPAPEFEGGPSVFLFPPKPKDTLMISRTPEVTCVVVDVSHEDPEVKFNWYVDGVEVHNAKTKPREEQYNSTYRVVSVLTVLHQDWLNGKEYKCKVSNKALPASIEKTISKAKGQPREPQVYTLPPSRDELTKNQVSLTCLVKGFYPSDIAVEWESNGQPENNYKTTPPVLDSDGSFFLYSKLTVDKSRWQQGNVFSCSVMHEALHNHYTQKSLSLSPGK

SEQ ID NO: 26 - protein, 357 aa, synthetic construct
  source 1..357: note = 1-G07-FCWT
QVQLVESGGGKAQPGGSLRLSCVASRITFRHYDLSWYRQAPGQERELVATVTNGGVITYADSVKGRFTISRDNAKNTVQLQMNNLKPEDTAVYYCNAVWVYLQRLTQNKKENDYWGPGTQVTVSSEPKSSDKTHTCPPCPAPELLGGPSVFLFPPKPKDTLMISRTPEVTCVVVDVSHEDPEVKFNWYVDGVEVHNAKTKPREEQYNSTYRVVSVLTVLHQDWLNGKEYKCKVSNKALPAPIEKTISKAKGQPREPQVYTLPPSREEMTKNQVSLTCLVKGFYPSDIAVEWESNGQPENNYKTTPPVLDSDGSFFLYSKLTVDKSRWQQGNVFSCSVMHEALHNHYTQKSLSLSPGK

SEQ ID NO: 27 - protein, 209 aa, synthetic construct
  source 1..209: note = 1-G07-ABD
QVQLVESGGGKAQPGGSLRLSCVASRITFRHYDLSWYRQAPGQERELVATVTNGGVITYADSVKGRFTISRDNAKNTVQLQMNNLKPEDTAVYYCNAVWVYLQRLTQNKKENDYWGPGTQVTVSSGGGGSGGGGSGGGGSQHDEAVDANSLAEAKVLANRELDKYGVSDYYKNLINNAKTVEGVKALIDEILAALPAAACAAAHHHHHH